European Patent Application EP 4 813 404 A1, published September 30, 2026. Title: 睡眠改善剤. Applicant: 国立大学法人富山大学. The sequence listing filed with the application follows.

SEQUENCE LISTING (3 sequences)

SEQ ID NO: 1 - protein, 31 aa, Rattus norvegicus
AGAELEPYPCPGRRCPTATATALAPRGGSRV

SEQ ID NO: 2 - protein, 31 aa, Mus musculus
AGAELEPHPCSGRGCPTVTTTALAPRGGSGV

SEQ ID NO: 3 - protein, 31 aa, Homo sapiens
AGAEPAPRPCLGRRCSAPAAASVAPGGQSGI